European Patent Application EP 4 706 387 A1, published March 11, 2026. Title: Methods for determining the sex of birds, birds, method of production, egg populations, and sex determination apparatus. Applicant: 株式会社セツロテック. The sequence listing filed with the application follows.

SEQUENCE LISTING (4 sequences)

SEQ ID NO: 1 - DNA, 1632 bp, Gallus gallus domesticus
  source 1..1632: mol_type = genomic DNA
atgaccctaacggaacagcacttccaggagtctcctccacccccttctgaggtggccaaggcagacatggacagcacaggagggaaggagaaggctgcgcagccctccacggcaaggactggagcgctggtgcgcaagcagcaagcaacgggaaggctgatcatgcacagcatggcgatgttcgggagggagttctgctatgctgtggaggctgcctttgtcacgccagtgctgctcagtgtagggctgcccaagagcctgtacagcctggtgtggctcatcagccccatcctgggcttcgtgctgcagcccgtggtaggttctgccagtgatcactgcgcctgtagctggggcaggaggcgaccttacattctgggtctgggcatcataatgctggtaggaatggctttgtacctcaatggggacgagatgatctcagctttcatcggtgagagagagaagcaacggacatgggcaatagtcattaccatgctgggagtagtgctttttgattttgcagctgactttattgatggccccatcaaagcatatttatttgacgtctgctctcatgaagataaagagaagggtctgcattatcatgccctgtttacaggcttaggaggagcactgggctacctgacaggtgctgtggactggggtgaaactgtactaggatattccttgacgtcagaattccaggtgattttcctcttgtcagccttggttttcctcatctgccttattgtacatctacgcagtattcctgaagtcccactcagatatggcaacaaagagacaaagctcttgttggaagtgaccgagccctataagtacagatccatagaggaaatcaagaatggatactcgtcatgtactgacttaaatgctacgagtaagacaaagaaaggtactgatgcatcgtgttcagaggctcaaaggcggatgacacttaagtcactcttgaagactcttttaagcatgccatcccattatcgctgtctgtgtgtgagccacctctttggatggatggctttcatgtccaacatgctcttcttcacggatttcatggggcaggttgtgtaccagggcagtccttatgcttctcataactccacactataccatacctacagaagaggagtggaggttggatgctgggggctgtgcatcaatgcgattgcatcctcagcctattcttacctgcagaaagtccttctgccatacataggattaaagggactttatttcattggatacctactttttggattaggcactgggttgattggcttgtttcccaatgtctattccaccttggttctatgttcgctttttggagtcatgtccagcactctgtacacagtgcctttccaactcattgcagagtatcacaaagaagaagaggacctgaatctgcagcagaaggaacaaggcacagagcatgggagaggaaagggcattgactgtgctgctctcacctgcatggtccagctggcacagatcattctcggtgtgggcctagggctcttggtcagtgttgctggcagtgcggtcactgtgatttcagcatcaatggtggcactgattggctgctgctttgttgctttctgtgttcgatatgtggggtaa

SEQ ID NO: 2 - protein, 543 aa, Gallus gallus domesticus
MTLTEQHFQESPPPPSEVAKADMDSTGGKEKAAQPSTARTGALVRKQQATGRLIMHSMAMFGREFCYAVEAAFVTPVLLSVGLPKSLYSLVWLISPILGFVLQPVVGSASDHCACSWGRRRPYILGLGIIMLVGMALYLNGDEMISAFIGEREKQRTWAIVITMLGVVLFDFAADFIDGPIKAYLFDVCSHEDKEKGLHYHALFTGLGGALGYLTGAVDWGETVLGYSLTSEFQVIFLLSALVFLICLIVHLRSIPEVPLRYGNKETKLLLEVTEPYKYRSIEEIKNGYSSCTDLNATSKTKKGTDASCSEAQRRMTLKSLLKTLLSMPSHYRCLCVSHLFGWMAFMSNMLFFTDFMGQVVYQGSPYASHNSTLYHTYRRGVEVGCWGLCINAIASSAYSYLQKVLLPYIGLKGLYFIGYLLFGLGTGLIGLFPNVYSTLVLCSLFGVMSSTLYTVPFQLIAEYHKEEEDLNLQQKEQGTEHGRGKGIDCAALTCMVQLAQIILGVGLGLLVSVAGSAVTVISASMVALIGCCFVAFCVRYVG

SEQ ID NO: 3 - DNA, 71 bp, Gallus gallus domesticus
  source 1..71: mol_type = genomic DNA
aagcatatttatttgacgtctgctctcatgaagataaagagaagggtctgcattatcatgccctgtttaca

SEQ ID NO: 4 - DNA, 25 bp, synthetic construct
  source 1..25: mol_type = other DNA; note = gRNA for chicken SLC45A2 gene
tttgacgtctgctctcatgaagata